European Patent Application EP 4 265 297 A1, published October 25, 2023. Title: COMPOSITION FOR IMPROVING INFLAMMATION OF BRAIN TISSUE. Applicant: MEIJI CO., LTD. The sequence listing filed with the application follows.

SEQUENCE LISTING (1 sequence)

SEQ ID NO: 1 - DNA, 533 bp, Lactobacillus plantarum
ttaaagctggcggcgtgcctaatacatgcaagtcgaacgaactctggtattgattggtgcttgcatcatgatttacatttgagtgagtggcgaactggtgagtaacacgtgggaaacctgcccagaagcgggggataacacctggaaacagatgctaataccgcataacaacttggaccgcatggtccgagtttgaaagatggcttcggctatcacttttggatggtcccgcggcgtattagctagatggtggggtaacggctcaccatggcaatgatacgtagccgacctgagagggtaatcggccacattgggactgagacacggcccaaactcctacgggaggcagcagtagggaatcttccacaatggacgaaagtctgatggagcaacgccgcgtgagtgaagaagggtttcggctcgtaaaactctgttgttaaagaagaacatatctgagagtaactgttcaggtattgacggtatttaaccagaaagccacggctaactacgtgccagcagcccgcgggtctcta